European Patent Specification EP 3 543 253 B1, published March 27, 2024. Title: MICE EXPRESSING HUMANIZED T-CELL CO-RECEPTORS. Applicant: Regeneron Pharmaceuticals, Inc. Application EP. The sequence listing filed with the application follows.

SEQUENCE LISTING (59 sequences)

SEQ ID NO: 1 - DNA, 202 bp, Artificial
  synthetic
aggggaaacccgcaaaggatgggacatagggagacagctgttaacatctgaaacatgaccttcttttctgtgcagcacaactcctagctgtcactcaagggaagaaagtggtgctgggcaaaaaaggggatacagtggaactgacctgtacagcttcccagaagaagagcatacaattccactggaaaaactccaaccagat

SEQ ID NO: 2 - DNA, 240 bp, Artificial
  Synthetic
ctggtcacctggatgaagtgagggagggccctctgggtttggggctggttttgaactgagacatccatgagccagcctggggctggcttcactgaagatcatctatgtcgggtgcggagaaagaggtaatgaaatggcacatgctatgtacaaactctattgctgagcagcacccagtcctgagctggctctgaattgagggtgaaattcacacattctcccccaacatctataatctgg

SEQ ID NO: 3 - DNA, 18263 bp, Artificial
  Synthetic
  misc_feature (2957)..(2957): n is a, c, g, or t
  misc_feature (3193)..(3193): n is a, c, g, or t
aagaaagtggtgctgggcaaaaaaggggatacagtggaactgacctgtacagcttcccagaagaagagcatacaattccactggaaaaactccaaccagataaagattctgggaaatcagggctccttcttaactaaaggtagggttgcctggctccccatccagggaggaaaacacactatggagtgaaagcctttggtgtctgagatctggtcttagttaaactctgggatcggcgcgccgaattcctgcagcccgggctcgagataacttcgtataatgtatgctatacgaagttatatgcatccgggtaggggaggcgcttttcccaaggcagtctggagcatgcgctttagcagccccgctgggcacttggcgctacacaagtggcctctggcctcgcacacattccacatccaccggtaggcgccaaccggctccgttctttggtggccccttcgcgccaccttctactcctcccctagtcaggaagttcccccccgccccgcagctcgcgtcgtgcaggacgtgacaaatggaagtagcacgtctcactagtctcgtgcagatggacagcaccgctgagcaatggaagcgggtaggcctttggggcagcggccaatagcagctttgctccttcgctttctgggctcagaggctgggaaggggtgggtccgggggcgggctcaggggcgggctcaggggcggggcgggcgcccgaaggtcctccggaggcccggcattctgcacgcttcaaaagcgcacgtctgccgcgctgttctcctcttcctcatctccgggcctttcgacctgcagccaattgttgacaattaatcatcggcatagtatatcggcatagtataatacgacaaggtgaggaactaaaccatgggatcggccattgaacaagatggattgcacgcaggttctccggccgcttgggtggagaggctattcggctatgactgggcacaacagacaatcggctgctctgatgccgccgtgttccggctgtcagcgcaggggcgcccggttctttttgtcaagaccgacctgtccggtgccctgaatgaactgcaggacgaggcagcgcggctatcgtggctggccacgacgggcgttccttgcgcagctgtgctcgacgttgtcactgaagcgggaagggactggctgctattgggcgaagtgccggggcaggatctcctgtcatctcaccttgctcctgccgagaaagtatccatcatggctgatgcaatgcggcggctgcatacgcttgatccggctacctgcccattcgaccaccaagcgaaacatcgcatcgagcgagcacgtactcggatggaagccggtcttgtcgatcaggatgatctggacgaagagcatcaggggctcgcgccagccgaactgttcgccaggctcaaggcgcgcatgcccgacggcgatgatctcgtcgtgacccatggcgatgcctgcttgccgaatatcatggtggaaaatggccgcttttctggattcatcgactgtggccggctgggtgtggcggaccgctatcaggacatagcgttggctacccgtgatattgctgaagagcttggcggcgaatgggctgaccgcttcctcgtgctttacggtatcgccgctcccgattcgcagcgcatcgccttctatcgccttcttgacgagttcttctgaggggatccgctgtaagtctgcagaaattgatgatctattaaacaataaagatgtccactaaaatggaagtttttcctgtcatactttgttaagaagggtgagaacagagtacctacattttgaatggaaggattggagctacgggggtgggggtggggtgggattagataaatgcctgctctttactgaaggctctttactattgctttatgataatgtttcatagttggatatcataatttaaacaagcaaaaccaaattaagggccagctcattcctcccactcatgatctatagatctatagatctctcgtgggatcattgtttttctcttgattcccactttgtggttctaagtactgtggtttccaaatgtgtcagtttcatagcctgaagaacgagatcagcagcctctgttccacatacacttcattctcagtattgttttgccaagttctaattccatcagacctcgacctgcagccctagataacttcgtataatgtatgctatacgaagttatcctaggccagagggcttgggttgacagaaactcagtggcattcttatccagagtttctctacaccaactgctggtggcccagggaaaggtggtatgtgaatttcaatattttaatatttaatattcatgaacttattttagtgagttttagaacaatcactatcacttaaaacccgtgatttcttgagtattgttgctacagacctatgtagataatactttgcacagtgactcatatgtataatcctagcactgtgggaggctgaggccggaggattgcttgagtccaggagttcaagaccagcctgaacaacatagtgagactctgtctctatgaaaaaaaatatatatatattttttttggagacaaggtctagttctatcacccaggctccagtgcagtggtgtgatctcggctcactgcaatctccacctcccaggctcaagtcatcatcccacctcagcctcccaagtagctgggactacaggcatgcaccaccatgccaggctaatttttgtattttttatagagacagggtttcaccatgttggccaggctggtctcgaactcatgagctcaagtgatccactcaccttggcctctcagagtgctggaattacaggtgtgtgtcactatgcctagccaaaaaaaatttttttaattaaaaaaaaaaaggccggctgtagtggctcacacctgtaatccagaactttgggagtttgaggtgggcagatcaccggnggtcaggagttcaagaccagtctggccaacatggtgaaacccggtctctactaaaaatacaaaaattagccaggtgtgggggtgcagtcctgtacttccagctactcaggaggctgaggcaggagactcgcttgaacctgggaggcaaaggctgcagtgagctgagattgcaccactgcactccagcctgggtgacagagcaagacttcatctcaaaaaaaaaaaaaaagctgcanatttattattattattattagtttatttatttatttttttgagacagagtctcgttctgtcgcccaggctggagtgcggtggcgtgatcttggctcattgcaacctccacctcccgggttcaagtgattctcctgcctcagcctcccgagtagctgggactacaggcgtatgccaccatgcctggctaattttttgtacttttagtagagacagagtttcacggtgttagccaggctggtcttgatctcctgacctcgtgatttaccctccttggcctcccaaagtgctgggattacaggcgtgagtcactgtgcccggcccagaatcatttttttctacttttttttttttgaggcaaactctcgatctgttgcccaggctggagtgcagtgggcatgatcttggctcactgcaagctctgcctcccaggttcaagcaattctcctgcctcagcctcctgagtagctgggactacaggcgtgtgccaccatgcccggctaatttgcgtatttttagtagagaccggttttcatcatattggccaggctggtcttgaactcctgacctcaagtgattctcccaccttagcctcccaaagtgctgggattacaggcatgagctactgcacttggccttttctcctggttttaaaactattatatgctcattacaaaatatttggtcaatgaagaaaagaatatggaagaaaatcaaatgcatgcatacttctatcactcagagatatcctctgctaacattttgattgattttcttccaatctttttttttttttttctttttgagacagggtctcactctgctgcccaggctggagtacagtggcatgaccacaacacatcacagcctcaagtgatcttcccacttcagccttcccagtagctgggactacaggtgcacgccaccatgttcacctaattttttactttttgtagagatgagacttcaccatgttgctcaggctggtcttgaattcctaggctcaagtgatcttcccgctttggcctcccaaagtgctgggattataggtatgagccactgcatgtggcctattttcttccactgttgttcggcgtggagaatattatatacataattacgtaaatgatatcatactgtatataccttttttcctactccttccttaagttatatcataatgagactaccaattattagactttttttcttttttttgagacggagtctcggtctgtcacctaggctggagtgcaatggcgcgatctcagctcgctgcaacctctgcctcccaggttcaagcaattctgcctcagcctcccgagtagctgggactacagacacgtgccaccatgcccagctaacttttttatttttttattagagacagggttccaccatgctagcaggatggtctcaatctctcgacttcgtgatcagcccggcttggcctcccaaagtgctgggagtacaggtgtgagccaccgcactcggcctagactaactatttaaagtaatctggcaatgtttaacgaatacaaaactctaaaacccttggacctaataatagctattttggaaagtctacttgacagaaataaaattgtgaatattcttttttgttgtttttttgagacagagtctcatttggacgcctaggctggagtgcagtggcatgatctcggctaactgcaacctccacctcctgggttcaagtgattctcctgcctcagcctcctgagcagctgggattacaggtgtgcaccaccatgtctggctaatttttgcatttttagtagatggggtttcaccatgttgaccagggtggtctggaacttctaccctcaagtgatctacccaccttggcctcccaaagtgctgggattacaggtgtgagccaccacgcctgaccagtgaacacttaataatatctatggaaaggtgttattataagaattgcttgtggggccgggcgtggtggctcacgcctgtaatcccagcactttgggaggctgtggcaggcggatcacgaggtcaggagatcaagatcatcctggctaacacggtgaaaccccgtctctactaaaaataccaaaaaattagccaggcgtggtggcgggcacttgtaatcccagctatccaggaggctgaggcaggagaattgcgtgaacccaggaggcggaggtcgcagtgagctgagaccgtgccattgcactccagcctgagtgacagagtgagactccatcacaaaaaataaataaataaataaataaaatataaataagtaaataaaggtcaggagtggtggctcacgcctgtaatcccagcactttgggaggccgaggtggacagatcatgaggtcatgagatcaagaccatcctggctaacacagtgaaaccctgcctctactaaaaatacaaaaagtcatccaggtgtggtggcacacacctatagtcccagctacttgggaggctgaggcaggagaatcacttgaacccaggaggcagaggttgcagtgagctgagatcgcgccactacactccagcctaggcgacagagcaagactctgtctcaaaataaataaataaataaataaataaataaataaataaataaaataaaaagcacacacacacacacacacacacacacacaatgcaaaagacccaccctactacaactaacattatatttaatggtgaaaaactgaattctttctccctaagtgcaggaataagacaaagatgtctgctcttactactcttattcaacataatactgcaatcccttgccagtgcaataaggcaagaaaaatgaaataaaaggaaaactgatcagaaagaaagaaataaaactgttcctatttgtggatgacatgattacatagaaaatctcaaagaatctgtaagaaacttcttagaattaataaatgaattcatcaaggttgcagaatataagataaacataaaaaatctattgtatttctatatattagcaaggaacatgtgtacacagaaattaaaactacaataccatttataattgctcaaaaaggccaggcatggtggctcacacctgtaattcctgcactttgggaggccaaggtgggaagattgcttaagcccaggagttcaagaccagcccgggcaacatagtgagaccttgtctctacaaaaagtaaaaaattagctgagcatggccgggtgcagtggctcactcctgtaaccccaacactttgggaggctgaggcgggcggatcatgaggtcaggagatcgagaccatcctggctaacacggtgaaaccctgtctctactaaaaacacaaaaaattagctggatgtggtggcaggcgcctgtagacccagctactcgggaagctgaggcaggagaatggcgtgaacctgggaggcggagcttgcagtgagctgagattgtgccactgcactccagcctgggtgacacagtgagactacgtctcaaaaaaaaaaaaaaaaaaattagctgagcattatggtgtatgcctgtagtcccagctactggggaggctgaggtgggaggattgcttgagccctaggagggcaaggctgcagtgagccatgatcacaccactgctttccagcctcggtaggagagcaagaccctatctcaaaaaaaaaaaaaaaaaaaaaagaaaagaaaagaaaagaaaagaaaaagaaagagagaaagaaatacttaggtgtaaatctaaaaaacatgcgtagggccaggtgcagtggctcatgcctgtaatcccagcactttgggaagttgaggctggcggatcacttgaagtcgggagtttgagaccagcctggccaacatggtgaaaccccgtctctactaaaaatgcaaaaattaggcaggtgttgtggcgcatgcctgatcccagctactttggaggctgaggcaggagaattgcttcaacccgggaggcagaggttgcagtgagccaagactgttccactgcactccagcctgggcaacagagtaagagtctgtctcccgaaaaaaaaaaaaagaaaaaagaaagcattgaattgtatgctaaaaactacacgatgctgattaaagaagtcaaagaagatctaaatatatggagagacatgctgtactcatggattgatggattggaagactcaacataagacagatatcaattttccccaaattaatatacaagtttaatccaattcctataaaaataccagcaagattttttgtagatataaacaagttggccaggtgtagtggcttacacctgtaatcctagcactttgggaggctgaggtgggaagatcgcttgagcccaggtgttcacgactgcagtgagctatgattgtgtcactgcattccagctggcactccagcctaagtgacaaagggagaccctgtctcaaaaacaaaaacaaaaccaaaataattttgctctgcaaaatccctattaagaagaagaaaagaggctgggcacagtggctcaccgctgtaatcccagcacgttgggaggctgaggcaggctgatcacttcagcccagaagtttgagatcagcctgggcaacatgaggaaaccccgtctctaccaaaaaaaaaaaaaggtacatacacacacacacacacacacacacacatacacaagtatatacacatatatatacacatacaggtgaatagatgtatatacatctatttattgtgaatatacatctatacacacacgtgtgtgtacacatatatttaaaatttatttttatttatttatttatttttgagacagagtcttgctctgtcacccaggctgggtgcacctgtattcccaacgacacaggaggctgaggtgggagaatcactgagccagggaggcagaggttgcagtgagccaagatgttgcctggttgcctgggcaacagagcgagaccctatatcaaaaaagaagaataataagaaaagacagtttacagaatataagaaaatatattcacaatccacatacttagcaaaggactggtatctagaatatgataaacaactctcaaaactcaaaaccaaaaaaatgaacaattcaattagaaaacaggccgaaaaggacatacagttggcaaataagcacatgaaaagttgttcaacatcattaatcattagggatatgtacattaaaaccacaataggctatcactaaacctatcagaatggctaaatacaaaattggaacaccaccaaatgctgatgaggatgtggagaaactgggtcattcttccaatattggtgggaggctaaaatggcaaagccactctggaaaacagtttgatagtttcttataaaacaaaacatgcggccgggcgcggtagctcacgcctgtaatcccagcactttgggaggccgaggcgggtggatcacgaggtcaggagatcgagaccatcctggctaacacggtgaaaccctgtctctactaaaaatacaaaaaattagccgggcgtggtggcgggcgcctgtagtcccagctactcgggaggctgaggcaggagaatggtgtgaacccgggaggcggagcttgcagtgagccgagatcgcgccattgcactccaacctgggagacggagggagactccgtctcaaaaaaacaaaaacaaacaaacaaaaaacatgcaacaatccagcaatattgcacccctaggcatttatcctagagcaatgaagacttatgcccacacaaaaagctgcacacaaatgttcatagcagctttattcatggtagccaacaattagaaacaatctagatgtccttcaactggtgaatgattacatccataccacgaaatacttttcagcaataaaaaggatgaatcatagtacacaccacaacctggatgaatctccagggaattatgctgagtgaaaaaaagccaatctcaaaaggtaatatactgtattaatccatttatataacattcttaaaataactaattatagaaatggagaacagatgagtgattgccaggggttaaggggctcagggatggggaggggaaggggtatggctacaaaaagcaacaaccttatggcgccggaaatgttctgtattctgattgtgtcaatgtgagcatactggttgagatatagtgctacagttttgcaagttattaccatcagagtaaactggatagagggcacataggatttctctgtattacttcttacaactgcaagtgaatctacaattatctcaaaataataagtttagtttaatgctaggcgtggtggctcacatctgtaatctcagctctttgggaggctgagacgggtggatggcttgagtccaggagttcgagaccagcctggccaacatggcaaaaccggtctctactaaaaatacaaaaattagctgggcgtggtggcaagtgcctgtagtcccagctactcgggaggctgaggcaggagaattgcttgaacccgggaggtggaggttgcagtgagccgagatcacgccactacactgtagcttgggcgacagagtgaggctctttctcaaaaaaaaaaaaaaaaaaaaaaaagcaggcaggcagggccaggaaagcgtataatttttgtagttcaaatgactaacctaaaaagtgaagattggccaggcgcagtggctcacgcctgtaatcccagcactttgggaggccaaggcgggtggatcacgaggtcaggagattgagccactctggctaacacagtgaaaccccgtctctactaaaatacaaaaaattagctgggcgtggtggcacccgcctgtagttgcagctacttgggaggctgaggcaggagaatcacttgaacccaggaggcgaagttgcagcgagccgagatcacactactgcactccagcctgggtgacaaagtgagattctgtctcaaaaaaaaaaaaaaaaaaaaaaaaaaaaaaaagtgaagtttacctttttttttaaatttttcttcttttccttccctactttgtgagataattttcttctttttaaaaagccaagagcttacttctgtaagtaaagattatcttaagacaacttagaaatgtatattattagtattttctatttcattgtaagttatttgtaaatattggttttggtgctaacctagaattccatcaaattaattgtcccctaatatatggccattatcattttgtctaacattgtatcctattaacaatgctgtaagtattatttttgtagctaaattatggtttgcattttaaaattattgttttaaggataaagttccagaaatgaaattaaggatatgaactttttgagcacatcttgtcagcactgagtagtattatttaaaacttttggggggggcaattttataattgaaaaatatatcattgttttaatttgcatttctttcactgcctatgagattaaaacaatgcactactttccaaaaattcttaagtcttttgtgttgatgcttttgttctgtttctatggatctcatcttccttcagaacagctccccttcccaacttcctgatttctaacaataacagtatcaccctccttgttctcccaatttctgaaacacagagtcatgtttttttctctgcttcaatccctggtttcctatcgtcatcaattatgacctttccttgctttgaaagtgttttgggccgggcatgatgtctgccacctattgtaatcctagcactttgggaggctgaggcggctggatgacttgacctgaggatttcgagaccagcctgggcaacagggcgaaacctcgtctctacaaaaaatacaaaagttagtcgggagtggtggcacatgcttgtagtcccagttacttggggggctgaggtggcaggatctcttgagcccacgaggtagatgttgcagtgagccgtgattgcgccactgcaccccagcctaggtgacagagtgagaccctgtctcaaaaaaaaaaaaatgttctagtttcttcctcttctttgttcccatgggaatgccaccatcaccagccaaggctcacatacctcccacctggattacagtgagcttccaggtaatttggtctgctactagtctcgcctacttggatttcccttccccctgctgcagcattgccttccaaagccatgctttgcacatgccacatcctagcccattagactaagcctagaagcctctgcaggacgttcaccctctcagcgccactgctcagtttcccagtggaaacctctgcacccaggaggtttccccacagcttgcctgtgctgcctctctggagcttttctcccttcctgtaatgtccttgctgctccccgtctctagtccattgcctatacctctttttttttttttttttgagatggagtctctctctctcatccaggctggagtgcagtggcgcgatctcggctcactgcaacctttgtctcctgggttcaagggattctcctgcctcagcctcccgagtaactgggattacaggcgtgcaccaccattcctggctaatttttgtatttttagtaaagactgggtttcaccatgttggccaggctggtcttgaactcctgccctcaggtgatccacctgcctcggcctcccagagtgctgggattacaggcgtgagccaccgcacctgccacaggcccatacctcttttaagtcttcattcaataccagttgtcccatgaatttgtcccagactcactcatatgcttagacctttcatattatcttgccatagctttttcaaagtatgggacagcatggacaagcaggccatggttttcttttgaagagaagcaaggaggcagagttattttaggaggagggttatacatttcattttgaaccaattgcgtttggggtgatggcaggatattaacataaacttatttcttggaccattggaaatgtgtgcctagaactgaggagagaggtcagggctggcagtaacaacttggccacaatctgcagagctgactggggatgaggtggaatttagaatgtctgtagaaacggggaagagaaccaaagacagagtctgggacaacacctaaatgtagatgtcagagcaagagttcaagacgaagaaaaacgaatcatacttagaaatggaggggaggaacaaaagaggcggagcaaagtggggcagaaccagagtaggccacgcttttaagaagtttggtaaaggaactgtgaaaggaatgtagttgaatttcagggtaagctggggaattaaagcagtgtgtagatccagggcaaacagcaagtagggcaggaaccactgaaggaacaaataaagggggaggttgggtccaggttgtcttgagtagggaagtttttttaaaaagtgtgaaactgaaggtgtggggtggattgggtgcctgccgtgctctgaggaagcttggggcaactgtgtgctgaggctgtgaggttgtctggaaggggctcctggacagtaagagctgagcagtggggaagaggactgtgtggtctggaagaggagagaaaggagagtgagtgactgaactggtatccaggctcccacaccaaggcagaaagagggagaggacctgggcatctcagggaggcagaggcagtaccaagcagggtgagaggctttagtcttagccacctttgccccattcctccaaatatacattctaagtaaaaacaaaacaaaacagaactgtttgctatgtaaatttagcttctaaagccctgttctacagagattttggagcttccactgcacccagaaaatgcacagctaaagagaaaacttcccttggtgatggttattagattttacaagaagaggccaaaggagacacatacttatgccagaagaactttccagagatagcattgcatagcgaaatagcctgaattatttttattttttaaaacattttttcttttcttttttcttttctttttctttttttttttttttttttgagacagagtctcactctgtcacccaggctggagtgcagtggcgtgatcttggctcactgcaatctccacctcccgggttcaagccattctcctccctcagcctcccaagtagctgggattacaggcatgcgtcactatgctctggctaattttttttttctttttttttttggtatttttagtagagatggggtttcaccatgttggccaggctggtcttgaactcctgacctcaagtgatccaccgccttggcctcccaaagtgctgggatttcaggcgtgagccaccgcacccggccaaaaatttcttttctttaagatgaggcctcactctgttgcccaggctggagtgcagtgttacaatcatagctcactgtaactttgaactcctgggctcaagtgatcctcctgcttcagcctctcaagtagctgggattacaggcatgtgccaccacacccagctaattttttttaaaataattttttttagagacgagggtctcgattggctgcctaggttggtcccagactcctgacgggctgcattttaatcctagctccaccacttacgggagtcaaaattcaaaagatagaaaagggcatataggctgggtgcagtggctcacacctgcaatcccagcaatttgggaggctgaggtgggcgggttgcttgaggtcaggagttcgagatcagcctgggcaacatggcaaaacttgtatctactaaaaatacaaaaattagccagatgtggtggtgtacacctgtaatcccagctactccgaaggctgaggcaagagaatcccttgaactcaggaggcagaggttacaatgagcagagatcgaacactcgactccataaaaacaaacaaacaaaaaaagaaagcaggctgggtgtggtggctcacgcctgtaaccccagcacttcgggaggccaaggcgagcggatcacctgaggttgggcattcgagaccagcctgaccaacaaggagaaaccctgtctctactgaaaatacaaaattagccgggcttggttgcgcatgcctgtaatctcagctactcgggaggcagaggcaagataattgcttgaacccgggaggcggaggttgcggtgagccaagatcatgccattgcactccaacctgggcaacaatagcgaaactccatctcaaaaaaaaaaaagcaaagggcatatagtgaaaagctttcttcctacacatgagtattcacttcctcttcctagaggcaaccaaggttatttttgtgtgtgtgtgtgtgtgtgtgtgtgtgtgtgtgtgttttgggacagtctcactctctcaccaaggctggaatgcagtggtgcgatctcactgcaaactctgcctcccagtctcaagcgatcttgtgcctcagcctcccagtttttttttcttttaaatggggtctcattctgtcgcccagggtggagtgcagtggcatgatcatagctcactgcagcctcgacctcctgggtcaggttatcctcccacctcagcctccggcatagctggggctactggcatgcaccaccacactcagttaattttttttcttttttgagacagagtctcactctgtcacctagactggagtgcagtggtgccatctcatttgtttcactgcaacctttgacttctgggctcaagtgattctcccacctcagcctcccaaggcggctaattaaaaaaaatttttttttttttttttttagagatggggtttcgccatgttgcccaggctgatctcgaactcctgggcacaaacaatctttccacctcgatctttcaaagagctgggatgagagatttccaccatgcctggcctcattttcttttttaatttttttttagacattatagctctttttaatggcctcattttcttatgtttaattcgagaattattcttttcatatacaaagaatatattttctccacctttaaaaacaaatagtagactgtttaacatctcgctttattcagttagtgatgtttcttagatacgggtccaaattagtacacaaagcacttcctcattcctctcttacggctgcatagcagtccactgaatgggtgagctatgatctatttaacctattctttattgatggacatttggttttgtatatacatttgtaattctgtatagattacaaatcaccatccaaagaaattgtactggtttattctcctacaatgtgtgagagttgggtaattacttaatctcaatatgtgagagtttaggcagttacctaatctctctgagtctcagtttctctatctgcaaaataaacaaaacagtgttgacagtatctatttctcggaattattgtggagattactgagatgatgcctgtaaagtatttggcatgtaggagttggtgctctccaaataaggatatgattttatttgtatttgtgagctactgtcccagccaggtaaatggatatgatgagacctccttgccagaccgggtttctctgattagaacgaggagcagatgttgcaggaaattagcaactgatatcagaagagccgtgggcattctcttgccagaggtgccctgtctccagggcgcctcagtccccccccatatgtcttctgctcccaggtccatccaagctgaatgatcgcgctgactcaagaagaagcctttgggaccaaggaaactttcccctgatcatcaagaatcttaagatagaagactcagatacttacatctgtgaagtggaggaccagaaggaggaggtgcaattgctagtgttcggatgtgagtggggcaggtggggatgaggatacctcctgcctggttcccttccccactactcccacccctgcaccaaatccagcctgagctggtgataccgcagcagccccaagaggaccaggctgtcaaactggcctccaaatgtcttaaaacccttcttgatcaggtgagggatgctggtgggcggaggagggaagaggccttgggaaaaggaaagaaaagggaaggaggcaagggaaggagggagagagactggggaagagaggatgaggggagaggaggaaagaagagagagaggaggggagagggaaaccctatcttggctgggggtgcgcagctgggtgctgggaggaaggagatgttgggacggcgataatggagagatgttgttggtttcctgttgtctgcccttctccttggggatggtatgtgtgtgacacagctggcctttccctccacagtgactgccaactctgacacccacctgcttcaggggcagagcctgaccctgaccttggagagcccccctggtagtagcccctcagtgcaatgtaggagtccaaggggtaaaaacatacagggggggaagaccctctccgtgtctcagctggagctccaggatagtggcacctggacatgcactgtcttgcagaaccagaagaaggtggagttcaaaatagacatcgtggtgctaggtaagggaagcccctcttcgcgcagtctcctccctgccccaggggctgacagcccctccctctgctctgactgccctgtttctggttctggtgctgggaggtcaggagtggagaagactaggtcccctagagctgaggcctgtcttgaaggactcactggggccctcatcctcagggggctgattggcagccacccctcagtgtggtggacatggagaaaggaaaggctggggaaggtaaggatgctagaggcccgagtctcctttggaggccccaaaggaggaatgtcagggagcttactttctttgttgcctcagctccacacccctaccaagttggcaaatccacttactcagggacactaacaccagtaagccaaccctgatgatgttctatgttgtacctctggacctctaagccaggccactgtggggagaccaaggtcctaccccagatcctgtcccctgggtgcttatgtgacttaaggtagacataaggtagtgtgccagtttagtgcatgtacgctgattgaaatcctggttctgccacaaccatgtgaccttgggtgagttactaaacctctctgcaccttggtttcagcctctgtgaaatggggatgatgttaactgccatagtgactacctcgtattaagttgaggactgatatacgtaaggcactgaaaatggtgcctggcacagagtaagccctagttaagtgttcgctgttattttgtgaagggtgatgaatacgcctctaaggagtggaggccaaatggcttctgtggtccaggaatcctaaggacagcaaggatcccctgtggctgggctgctctgtgatggcttccgggaggagggaggtggcctgctgtaggaaaatgctgggtggaagaagggagagaaggctggagaggtaggaaggaactgaagtatctgaagtgacaaggtgggtgtctggactcgtcgggtccccttccatctccctgctgcctccacatgccaaccccactcgtgcaccctcatcttcctatctcctcacccagggtctctcccttcccacctccagctttccagaaggcctccagcatagtctataagaaagagggggaacaggtggagttctccttcccactcgcctttacagttgaaaagctgacgggcagtggcgagctgtggtggcaggcggagagggcttcctcctccaagtcttggatcacctttgacctgaagaacaaggaagtgtctgtaaaacgggttacccaggaccctaagctccagatgggcaagaagctcccgctccacctcaccctgccccaggccttgcctcagtatgctggctctggaaacctcaccctggcccttgaagcgaaaacaggaaagttgcatcaggaagtgaacctggtggtgatgagaggtgaggggccaggccagggaggggtgggcaggggaaggagttggaggggcctggcccagggctccctctgaggcaagccaggccccaagaggggatgcctaggccctggtcacctggatgaagtgagggagggccctctgggtttggggctggttttgaactgagacatccatgagccagcctggggctggcttcactgaagatc

SEQ ID NO: 4 - protein, 458 aa, Artificial
  Synthetic
MCRAISLRRLLLLLLQLSQLLAVTQGKKVVLGKKGDTVELTCTASQKKSIQFHWKNSNQIKILGNQGSFLTKGPSKLNDRADSRRSLWDQGNFPLIIKNLKIEDSDTYICEVEDQKEEVQLLVFGLTANSDTHLLQGQSLTLTLESPPGSSPSVQCRSPRGKNIQGGKTLSVSQLELQDSGTWTCTVLQNQKKVEFKIDIVVLAFQKASSIVYKKEGEQVEFSFPLAFTVEKLTGSGELWWQAERASSSKSWITFDLKNKEVSVKRVTQDPKLQMGKKLPLHLTLPQALPQYAGSGNLTLALEAKTGKLHQEVNLVVMRVAQLNNTLTCEVMGPTSPKMRLTLKQENQEARVSEEQKVVQVVAPETGLWQCLLSEGDKVKMDSRIQVLSRGVNQTVFLACVLGGSFGFLGFLGLCILCCVRCRHQQRQAARMSQIKRLLSEKKTCQCPHRMQKSHNLI

SEQ ID NO: 5 - DNA, 21 bp, Artificial
  Synthetic
gaagtgggtgtgccattcaga

SEQ ID NO: 6 - DNA, 24 bp, Artificial
  Synthetic
aaagctcagaagcagacagagtca

SEQ ID NO: 7 - DNA, 25 bp, Artificial
  Synthetic
ttccaaaagcctacagcaggcccag

SEQ ID NO: 8 - DNA, 21 bp, Artificial
  Synthetic
tcatctccccttcctgaacct

SEQ ID NO: 9 - DNA, 21 bp, Artificial
  Synthetic
cccagccacaagaagaagaaa

SEQ ID NO: 10 - DNA, 26 bp, Artificial
  Synthetic
cttcccccgcatccatttttctgttc

SEQ ID NO: 11 - DNA, 22 bp, Artificial
  Synthetic
ggtctcgaactcatgagctcaa

SEQ ID NO: 12 - DNA, 25 bp, Artificial
  Synthetic
ggcatagtgacacacacctgtaatt

SEQ ID NO: 13 - DNA, 27 bp, Artificial
  Synthetic
tgatccactcaccttggcctctcagag

SEQ ID NO: 14 - DNA, 25 bp, Artificial
  Synthetic
gtcagggagcttactttctttgttg

SEQ ID NO: 15 - DNA, 26 bp, Artificial
  Synthetic
tgttagtgtccctgagtaagtggatt

SEQ ID NO: 16 - DNA, 27 bp, Artificial
  Synthetic
ctcagctccacacccctaccaagttgg

SEQ ID NO: 17 - DNA, 142 bp, Artificial
  Synthetic
tgtttgcctgtgacatgaactcattgtgacacaaaccactgtgctaggggggatccactagtaacggccgccagtgtgctggaattcgccctcgcaagggccaggcatataagtacacaataaacaaatggcagctctctcc

SEQ ID NO: 18 - DNA, 99 bp, Artificial
  Synthetic
cccctccttccttccccaggcactttccaagtgtcaactctagagcctatcgcggccgcaccggtataacttcgtataatgtatgctatacgaagttat

SEQ ID NO: 19 - DNA, 90 bp, Artificial
  Synthetic
ataacttcgtataatgtatgctatacgaagttatgtcgacgtagcctatttctctagatccaaaatgatgacaacaaaaggtaccttgtg

SEQ ID NO: 20 - DNA, 20 bp, Artificial
  Synthetic
gcagctctgccctcattcag

SEQ ID NO: 21 - DNA, 21 bp, Artificial
  Synthetic
catctttgccgtatggttggt

SEQ ID NO: 22 - DNA, 22 bp, Artificial
  Synthetic
ccccttcgtccctgctggttca

SEQ ID NO: 23 - DNA, 26 bp, Artificial
  Synthetic
caagaagactaccctgaagatgaaga

SEQ ID NO: 24 - DNA, 23 bp, Artificial
  Synthetic
tgtgagtgcaacaatggaaaact

SEQ ID NO: 25 - DNA, 22 bp, Artificial
  Synthetic
cgttcccccacccagagaccca

SEQ ID NO: 26 - DNA, 19 bp, Artificial
  Synthetic
ggcaccgagcagtgacagt

SEQ ID NO: 27 - DNA, 22 bp, Artificial
  Synthetic
ttcaccgtggatagtccctttt

SEQ ID NO: 28 - DNA, 24 bp, Artificial
  Synthetic
agttcctggccctctgggattccg

SEQ ID NO: 29 - DNA, 26 bp, Artificial
  Synthetic
ttgctttctttctgtagttgatttcc

SEQ ID NO: 30 - DNA, 21 bp, Artificial
  Synthetic
ccggcacactctcttcttgag

SEQ ID NO: 31 - DNA, 20 bp, Artificial
  Synthetic
tcccaccactgcccagccca

SEQ ID NO: 32 - DNA, 17 bp, Artificial
  synthetic
tgcggccgatcttagcc

SEQ ID NO: 33 - DNA, 18 bp, Artificial
  Synthetic
ttgaccgattccttgcgg

SEQ ID NO: 34 - DNA, 21 bp, Artificial
  Synthetic
acgagcgggttcggcccattc

SEQ ID NO: 35 - DNA, 100 bp, Artificial
  Synthetic
tgaacctgctgctgctgggtgagtcgattatcctggggagtggagaagctaggccgagccagttccgggtgtcgccgctggatcggacctggaacctggg

SEQ ID NO: 36 - DNA, 90 bp, Artificial
  Synthetic
atgccagggacagccctgatactgtaggtagagtcaagggctgtccaagtaccggtataacttcgtataaggtatcctatacgaagttat

SEQ ID NO: 37 - DNA, 89 bp, Artificial
  Synthetic
ataacttcgtataaggtatcctatacgaagttatctcgacctgatcttggagggagacctggaccgggagacgtgctgggggcagggtt

SEQ ID NO: 38 - DNA, 22 bp, Artificial
  Synthetic
gatgctcttggctcttccagaa

SEQ ID NO: 39 - DNA, 25 bp, Artificial
  Synthetic
atgaagccatatagacaacgaaggt

SEQ ID NO: 40 - DNA, 22 bp, Artificial
  Synthetic
ccagctccaaactcccccagcc

SEQ ID NO: 41 - DNA, 20 bp, Artificial
  Synthetic
tcagccccagagaccagaag

SEQ ID NO: 42 - DNA, 22 bp, Artificial
  Synthetic
tcaatcgcttgagagcacctaa

SEQ ID NO: 43 - DNA, 19 bp, Artificial
  Synthetic
ttgtcggccccgtggctca

SEQ ID NO: 44 - DNA, 17 bp, Artificial
  Synthetic
gcggttctcgggcaaga

SEQ ID NO: 45 - DNA, 20 bp, Artificial
  Synthetic
tcagggccgagcagaaatag

SEQ ID NO: 46 - DNA, 25 bp, Artificial
  Synthetic
acaccttcgtcctcaccctgagcga

SEQ ID NO: 47 - DNA, 22 bp, Artificial
  Synthetic
ggttcacctcaacctgttttcc

SEQ ID NO: 48 - DNA, 18 bp, Artificial
  Synthetic
cgcttccaggtgcgctaa

SEQ ID NO: 49 - DNA, 22 bp, Artificial
  Synthetic
acctgggccctgctttcaagcc

SEQ ID NO: 50 - DNA, 19 bp, Artificial
  Synthetic
ggtggagaggctattcggc

SEQ ID NO: 51 - DNA, 17 bp, Artificial
  Synthetic
gaacacggcggcatcag

SEQ ID NO: 52 - DNA, 23 bp, Artificial
  Synthetic
tgggcacaacagacaatcggctg

SEQ ID NO: 53 - protein, 210 aa, Artificial
  synthetic
MQPWLWLVFSMKLAVLHGNSVLQQTPAYIKVQTNKMVMLSCEAKISLSNMRIYWLRQRQAPSSDSHHEFLALWDSAKGTIHGEEVEQEKIAVFRDASRFILNLTSVKPEDSGIYFCMIVGSPELTFGKGTQLSVVDFLPTTAQPTKKSTLKKRVCRLPRPETQKGLTCSLTTLSLLVVCILLLLAFLGVAVYFYCVRRRARIHFMKQFHK

SEQ ID NO: 54 - protein, 243 aa, Artificial
  Synthetic
MASPLTRFLSLNLLLLGESIILGSGEARPSQFRVSPLDRTWNLGETVELKCQVLLSNPTSGCSWLFQPRGAAASPTFLLYLSQNKPKAAEGLDTQRFSGKRLGDTFVLTLSDFRRENEGYYFCSALSNSIMYFSHFVPVFLPAKPTTTPAPRPPTPAPTIASQPLSLRPEACRPAAGGAVKGTGLDFACDIYIWAPLAGICVALLLSLIITLICYHRSRKRVCKCPRPLVRQEGKPRPSEKIV

SEQ ID NO: 55 - DNA, 151 bp, Artificial
  Synthetic
tatggagtgaaagcctttggtgtctgagatctggtcttagttaaactctgggatcggcgcgccgaattcctgcagcccgggctcgagataacttcgtataatgtatgctatacgaagttatatgcatccgggtaggggaggcgcttttccc

SEQ ID NO: 56 - DNA, 151 bp, Artificial
  Synthetic
agtattgttttgccaagttctaattccatcagacctcgacctgcagccctagataacttcgtataatgtatgctatacgaagttatcctaggccagagggcttgggttgacagaaactcagtggcattcttatccagagtttctctacacc

SEQ ID NO: 57 - protein, 293 aa, Human
KKVVLGKKGDTVELTCTASQKKSIQFHWKNSNQIKILGNQGSFLTKGPSKLNDRADSRRSLWDQGNFPLIIKNLKIEDSDTYICEVEDQKEEVQLLVFGLTANSDTHLLQGQSLTLTLESPPGSSPSVQCRSPRGKNIQGGKTLSVSQLELQDSGTWTCTVLQNQKKVEFKIDIVVLAFQKASSIVYKKEGEQVEFSFPLAFTVEKLTGSGELWWQAERASSSKSWITFDLKNKEVSVKRVTQDPKLQMGKKLPLHLTLPQALPQYAGSGNLTLALEAKTGKLHQEVNLVVMR

SEQ ID NO: 58 - protein, 151 aa, Human
VLHGNSVLQQTPAYIKVQTNKMVMLSCEAKISLSNMRIYWLRQRQAPSSDSHHEFLALWDSAKGTIHGEEVEQEKIAVFRDASRFILNLTSVKPEDSGIYFCMIVGSPELTFGKGTQLSVVDFLPTTAQPTKKSTLKKRVCRLPRPETQKG

SEQ ID NO: 59 - protein, 152 aa, Human
RPSQFRVSPLDRTWNLGETVELKCQVLLSNPTSGCSWLFQPRGAAASPTFLLYLSQNKPKAAEGLDTQRFSGKRLGDTFVLTLSDFRRENEGYYFCSALSNSIMYFSHFVPVFLPAKPTTTPAPRPPTPAPTIASQPLSLRPEACRPAAGGA